European Patent Application EP 4 410 938 A1, published August 7, 2024. Title: Automatic dishwashing composition comprising a structural polypeptide. Applicant: AMSilk GmbH. The sequence listing filed with the application follows.

SEQUENCE LISTING (10 sequences)

SEQ ID NO: 1 - protein, 35 aa, synthetic construct
GSSAAAAAAAASGPGGYGPENQGPSGPGGYGPGGP

SEQ ID NO: 2 - protein, 35 aa, synthetic construct
GSSAAAAAAAASGPGGYGPENQGPCGPGGYGPGGP

SEQ ID NO: 3 - protein, 35 aa, synthetic construct
GSSAAAAAAAASGPGGYGPKNQGPSGPGGYGPGGP

SEQ ID NO: 4 - protein, 11 aa, synthetic construct
MASMTGGQQMG

SEQ ID NO: 5 - protein, 4 aa, synthetic construct
RGSM

SEQ ID NO: 6 - protein, 576 aa, synthetic construct
MASMTGGQQMGRGSMGSSAAAAAAAASGPGGYGPENQGPSGPGGYGPGGPGSSAAAAAAAASGPGGYGPENQGPSGPGGYGPGGPGSSAAAAAAAASGPGGYGPENQGPSGPGGYGPGGPGSSAAAAAAAASGPGGYGPENQGPSGPGGYGPGGPGSSAAAAAAAASGPGGYGPENQGPSGPGGYGPGGPGSSAAAAAAAASGPGGYGPENQGPSGPGGYGPGGPGSSAAAAAAAASGPGGYGPENQGPSGPGGYGPGGPGSSAAAAAAAASGPGGYGPENQGPSGPGGYGPGGPGSSAAAAAAAASGPGGYGPENQGPSGPGGYGPGGPGSSAAAAAAAASGPGGYGPENQGPSGPGGYGPGGPGSSAAAAAAAASGPGGYGPENQGPSGPGGYGPGGPGSSAAAAAAAASGPGGYGPENQGPSGPGGYGPGGPGSSAAAAAAAASGPGGYGPENQGPSGPGGYGPGGPGSSAAAAAAAASGPGGYGPENQGPSGPGGYGPGGPGSSAAAAAAAASGPGGYGPENQGPSGPGGYGPGGPGSSAAAAAAAASGPGGYGPENQGPSGPGGYGPGGPG

SEQ ID NO: 7 - protein, 576 aa, synthetic construct
MASMTGGQQMGRGSMGSSAAAAAAAASGPGGYGPKNQGPSGPGGYGPGGPGSSAAAAAAAASGPGGYGPKNQGPSGPGGYGPGGPGSSAAAAAAAASGPGGYGPKNQGPSGPGGYGPGGPGSSAAAAAAAASGPGGYGPKNQGPSGPGGYGPGGPGSSAAAAAAAASGPGGYGPKNQGPSGPGGYGPGGPGSSAAAAAAAASGPGGYGPKNQGPSGPGGYGPGGPGSSAAAAAAAASGPGGYGPKNQGPSGPGGYGPGGPGSSAAAAAAAASGPGGYGPKNQGPSGPGGYGPGGPGSSAAAAAAAASGPGGYGPKNQGPSGPGGYGPGGPGSSAAAAAAAASGPGGYGPKNQGPSGPGGYGPGGPGSSAAAAAAAASGPGGYGPKNQGPSGPGGYGPGGPGSSAAAAAAAASGPGGYGPKNQGPSGPGGYGPGGPGSSAAAAAAAASGPGGYGPKNQGPSGPGGYGPGGPGSSAAAAAAAASGPGGYGPKNQGPSGPGGYGPGGPGSSAAAAAAAASGPGGYGPKNQGPSGPGGYGPGGPGSSAAAAAAAASGPGGYGPKNQGPSGPGGYGPGGPG

SEQ ID NO: 8 - protein, 610 aa, synthetic construct
MASMTGGQQMGRGSMGSSAAAAAAAASGPGGYGPENQGPSGPGGYGPGGPGSSAAAAAAAASGPGGYGPENQGPSGPGGYGPGGPGSSAAAAAAAASGPGGYGPENQGPSGPGGYGPGGPGSSAAAAAAAASGPGGYGPENQGPSGPGGYGPGGPGSSAAAAAAAASGPGGYGPENQGPSGPGGYGPGGPGSSAAAAAAAASGPGGYGPENQGPSGPGGYGPGGPGSSAAAAAAAASGPGGYGPENQGPSGPGGYGPGGPGSSAAAAAAAASGPGGYGPENQGPSGPGGYGPGGPGSSAAAAAAAASGPGGYGPENQGPSGPGGYGPGGPGSSAAAAAAAASGPGGYGPENQGPSGPGGYGPGGPGSSAAAAAAAASGPGGYGPENQGPSGPGGYGPGGPGSSAAAAAAAASGPGGYGPENQGPSGPGGYGPGGPGSSAAAAAAAASGPGGYGPENQGPSGPGGYGPGGPGSSAAAAAAAASGPGGYGPENQGPSGPGGYGPGGPGSSAAAAAAAASGPGGYGPENQGPSGPGGYGPGGPGSSAAAAAAAASGPGGYGPENQGPSGPGGYGPGGPGSSAAAAAAAASGPGGYGPENQGPCGPGGYGPGGP

SEQ ID NO: 9 - protein, 1136 aa, synthetic construct
MASMTGGQQMGRGSMGSSAAAAAAAASGPGGYGPENQGPSGPGGYGPGGPGSSAAAAAAAASGPGGYGPENQGPSGPGGYGPGGPGSSAAAAAAAASGPGGYGPENQGPSGPGGYGPGGPGSSAAAAAAAASGPGGYGPENQGPSGPGGYGPGGPGSSAAAAAAAASGPGGYGPENQGPSGPGGYGPGGPGSSAAAAAAAASGPGGYGPENQGPSGPGGYGPGGPGSSAAAAAAAASGPGGYGPENQGPSGPGGYGPGGPGSSAAAAAAAASGPGGYGPENQGPSGPGGYGPGGPGSSAAAAAAAASGPGGYGPENQGPSGPGGYGPGGPGSSAAAAAAAASGPGGYGPENQGPSGPGGYGPGGPGSSAAAAAAAASGPGGYGPENQGPSGPGGYGPGGPGSSAAAAAAAASGPGGYGPENQGPSGPGGYGPGGPGSSAAAAAAAASGPGGYGPENQGPSGPGGYGPGGPGSSAAAAAAAASGPGGYGPENQGPSGPGGYGPGGPGSSAAAAAAAASGPGGYGPENQGPSGPGGYGPGGPGSSAAAAAAAASGPGGYGPENQGPSGPGGYGPGGPGSSAAAAAAAASGPGGYGPENQGPSGPGGYGPGGPGSSAAAAAAAASGPGGYGPENQGPSGPGGYGPGGPGSSAAAAAAAASGPGGYGPENQGPSGPGGYGPGGPGSSAAAAAAAASGPGGYGPENQGPSGPGGYGPGGPGSSAAAAAAAASGPGGYGPENQGPSGPGGYGPGGPGSSAAAAAAAASGPGGYGPENQGPSGPGGYGPGGPGSSAAAAAAAASGPGGYGPENQGPSGPGGYGPGGPGSSAAAAAAAASGPGGYGPENQGPSGPGGYGPGGPGSSAAAAAAAASGPGGYGPENQGPSGPGGYGPGGPGSSAAAAAAAASGPGGYGPENQGPSGPGGYGPGGPGSSAAAAAAAASGPGGYGPENQGPSGPGGYGPGGPGSSAAAAAAAASGPGGYGPENQGPSGPGGYGPGGPGSSAAAAAAAASGPGGYGPENQGPSGPGGYGPGGPGSSAAAAAAAASGPGGYGPENQGPSGPGGYGPGGPGSSAAAAAAAASGPGGYGPENQGPSGPGGYGPGGPGSSAAAAAAAASGPGGYGPENQGPSGPGGYGPGGPG

SEQ ID NO: 10 - protein, 1696 aa, synthetic construct
MASMTGGQQMGRGSMGSSAAAAAAAASGPGGYGPENQGPSGPGGYGPGGPGSSAAAAAAAASGPGGYGPENQGPSGPGGYGPGGPGSSAAAAAAAASGPGGYGPENQGPSGPGGYGPGGPGSSAAAAAAAASGPGGYGPENQGPSGPGGYGPGGPGSSAAAAAAAASGPGGYGPENQGPSGPGGYGPGGPGSSAAAAAAAASGPGGYGPENQGPSGPGGYGPGGPGSSAAAAAAAASGPGGYGPENQGPSGPGGYGPGGPGSSAAAAAAAASGPGGYGPENQGPSGPGGYGPGGPGSSAAAAAAAASGPGGYGPENQGPSGPGGYGPGGPGSSAAAAAAAASGPGGYGPENQGPSGPGGYGPGGPGSSAAAAAAAASGPGGYGPENQGPSGPGGYGPGGPGSSAAAAAAAASGPGGYGPENQGPSGPGGYGPGGPGSSAAAAAAAASGPGGYGPENQGPSGPGGYGPGGPGSSAAAAAAAASGPGGYGPENQGPSGPGGYGPGGPGSSAAAAAAAASGPGGYGPENQGPSGPGGYGPGGPGSSAAAAAAAASGPGGYGPENQGPSGPGGYGPGGPGSSAAAAAAAASGPGGYGPENQGPSGPGGYGPGGPGSSAAAAAAAASGPGGYGPENQGPSGPGGYGPGGPGSSAAAAAAAASGPGGYGPENQGPSGPGGYGPGGPGSSAAAAAAAASGPGGYGPENQGPSGPGGYGPGGPGSSAAAAAAAASGPGGYGPENQGPSGPGGYGPGGPGSSAAAAAAAASGPGGYGPENQGPSGPGGYGPGGPGSSAAAAAAAASGPGGYGPENQGPSGPGGYGPGGPGSSAAAAAAAASGPGGYGPENQGPSGPGGYGPGGPGSSAAAAAAAASGPGGYGPENQGPSGPGGYGPGGPGSSAAAAAAAASGPGGYGPENQGPSGPGGYGPGGPGSSAAAAAAAASGPGGYGPENQGPSGPGGYGPGGPGSSAAAAAAAASGPGGYGPENQGPSGPGGYGPGGPGSSAAAAAAAASGPGGYGPENQGPSGPGGYGPGGPGSSAAAAAAAASGPGGYGPENQGPSGPGGYGPGGPGSSAAAAAAAASGPGGYGPENQGPSGPGGYGPGGPGSSAAAAAAAASGPGGYGPENQGPSGPGGYGPGGPGSSAAAAAAAASGPGGYGPENQGPSGPGGYGPGGPGSSAAAAAAAASGPGGYGPENQGPSGPGGYGPGGPGSSAAAAAAAASGPGGYGPENQGPSGPGGYGPGGPGSSAAAAAAAASGPGGYGPENQGPSGPGGYGPGGPGSSAAAAAAAASGPGGYGPENQGPSGPGGYGPGGPGSSAAAAAAAASGPGGYGPENQGPSGPGGYGPGGPGSSAAAAAAAASGPGGYGPENQGPSGPGGYGPGGPGSSAAAAAAAASGPGGYGPENQGPSGPGGYGPGGPGSSAAAAAAAASGPGGYGPENQGPSGPGGYGPGGPGSSAAAAAAAASGPGGYGPENQGPSGPGGYGPGGPGSSAAAAAAAASGPGGYGPENQGPSGPGGYGPGGPGSSAAAAAAAASGPGGYGPENQGPSGPGGYGPGGPGSSAAAAAAAASGPGGYGPENQGPSGPGGYGPGGPGSSAAAAAAAASGPGGYGPENQGPSGPGGYGPGGPGSSAAAAAAAASGPGGYGPENQGPSGPGGYGPGGPGSSAAAAAAAASGPGGYGPENQGPSGPGGYGPGGPG